European Patent Application EP 4 814 020 A1, published September 30, 2026. Title: 通过重组反应制备异源多聚体的方法. Applicant: 江苏恒瑞医药股份有限公司. Application WO. The sequence listing filed with the application follows.

SEQUENCE LISTING (41 sequences)

SEQ ID NO: 1 - protein, 448 aa, synthetic construct
  CHAIN 1..448: note = Ipilimumab heavy chain
QVQLVESGGGVVQPGRSLRLSCAASGFTFSSYTMHWVRQAPGKGLEWVTFISYDGNNKYYADSVKGRFTISRDNSKNTLYLQMNSLRAEDTAIYYCARTGWLGPFDYWGQGTLVTVSSASTKGPSVFPLAPSSKSTSGGTAALGCLVKDYFPEPVTVSWNSGALTSGVHTFPAVLQSSGLYSLSSVVTVPSSSLGTQTYICNVNHKPSNTKVDKRVEPKSCDKTHTCPPCPAPELLGGPSVFLFPPKPKDTLMISRTPEVTCVVVDVSHEDPEVKFNWYVDGVEVHNAKTKPREEQYNSTYRVVSVLTVLHQDWLNGKEYKCKVSNKALPAPIEKTISKAKGQPREPQVYTLPPSRDELTKNQVSLTCLVKGFYPSDIAVEWESNGQPENNYKTTPPVLDSDGSFFLYSKLTVDKSRWQQGNVFSCSVMHEALHNHYTQKSLSLSPGK

SEQ ID NO: 2 - protein, 215 aa, synthetic construct
  CHAIN 1..215: note = Ipilimumab light chain
EIVLTQSPGTLSLSPGERATLSCRASQSVGSSYLAWYQQKPGQAPRLLIYGAFSRATGIPDRFSGSGSGTDFTLTISRLEPEDFAVYYCQQYGSSPWTFGQGTKVEIKRTVAAPSVFIFPPSDEQLKSGTASVVCLLNNFYPREAKVQWKVDNALQSGNSQESVTEQDSKDSTYSLSSTLTLSKADYEKHKVYACEVTHQGLSSPVTKSFNRGEC

SEQ ID NO: 3 - protein, 454 aa, synthetic construct
  CHAIN 1..454: note = CP11 heavy chain
EVTLKESGPVLVKPTETLTLTCTVSGFSLTRYGINWIRQPPGKGLEWLGVIWTGGDTNYNSALKSRLTISKDKSKSQVVLTMTNMDPVDTATYYCAREGVVNYYGSRYSFFDVWGQGTTVTVSSASTKGPSVFPLAPSSKSTSGGTAALGCLVKDYFPEPVTVSWNSGALTSGVHTFPAVLQSSGLYSLSSVVTVPSSSLGTQTYICNVNHKPSNTKVDKKVEPKSCDKTHTCPPCPAPELLGGPSVFLFPPKPKDTLMISRTPEVTCVVVDVSHEDPEVKFNWYVDGVEVHNAKTKPREEQYNSTYRVVSVLTVLHQDWLNGKEYKCKVSNKALPAPIEKTISKAKGQPREPQVYTLPPSRDELTKNQVSLTCLVKGFYPSDIAVEWESNGQPENNYKTTPPVLDSDGSFFLYSKLTVDKSRWQQGNVFSCSVMHEALHNHYTQKSLSLSPGK

SEQ ID NO: 4 - protein, 213 aa, synthetic construct
  CHAIN 1..213: note = CP11 light chain
DIQMTQSPSSLSASVGDRVTITCRASSSVSYMHWYQQKPGKSPKPWIYATSNLASGVPSRFSGSGSGTDYTLTISSLQPEDFATYYCQQWSSNPYTFGGGTKVEIKRTVAAPSVFIFPPSDEQLKSGTASVVCLLNNFYPREAKVQWKVDNALQSGNSQESVTEQDSKDSTYSLSSTLTLSKADYEKHKVYACEVTHQGLSSPVTKSFNRGEC

SEQ ID NO: 5 - protein, 97 aa, synthetic construct
  DOMAIN 1..97: note = Obscurin
SGAPRFLTCPKASVVSVGKDATLSSQIVGNPFPQVSWEKDKQPVTAGVRFRLAQDGDLYRLKILDLQLSDSGQYVSRARNAHGEAFACLGLQVDAEA

SEQ ID NO: 6 - protein, 98 aa, synthetic construct
  DOMAIN 1..98: note = Titin
GIPPKIECLPIDISIDEGKVLTVASCFTGEPTPEVTWSTGGRKIHSQEQGRFHIENTDDSTTLTIKDVQKQDGGLYTLTLRNEFGSDSATVNIHIRSI

SEQ ID NO: 7 - protein, 447 aa, synthetic construct
  CHAIN 1..447: note = CP11-Ip-F31-chain1
QVQLVESGGGVVQPGRSLRLSCAASGFTFSSYTMHWVRQAPGKGLEWVTFISYDGNNKYYADSVKGRFTISRDNSKNTLYLQMNSLRAEDTAIYYCARTGWLGPFDYWGQGTLVTVSSGGGGSSGAPRFLTCPKASVVSVGKDATLSSQIVGNPFPQVSWEKDKQPVTAGVRFRLAQDGDLYRLKILDLQLSDSGQYVSRARNAHGEAFACLGLQVDAEADKTHTCPPCPAPELLGGPSVFLFPPKPKDTLMISRTPEVTCVVVDVSHEDPEVKFNWYVDGVEVHNAKTKPREEQYNSTYRVVSVLTVLHQDWLNGKEYKCKVSNKALPAPIEKTISKAKGQPREPQVCTLPPSRDELTKNQVSLSCAVKGFYPSDIAVEWESNGQPENNYKTTPPVLDSDGSFFLVSKLTVDKSRWQQGNVFSCSVMHEALHNHYTQKSLSLSPGK

SEQ ID NO: 8 - protein, 211 aa, synthetic construct
  CHAIN 1..211: note = CP11-Ip-F31-chain2
EIVLTQSPGTLSLSPGERATLSCRASQSVGSSYLAWYQQKPGQAPRLLIYGAFSRATGIPDRFSGSGSGTDFTLTISRLEPEDFAVYYCQQYGSSPWTFGQGTKVEIKGGGGSGIPPKIECLPIDISIDEGKVLTVASCFTGEPTPEVTWSTGGRKIHSQEQGRFHIENTDDSTTLTIKDVQKQDGGLYTLTLRNEFGSDSATVNIHIRSI

SEQ ID NO: 9 - protein, 454 aa, synthetic construct
  CHAIN 1..454: note = CP11-Ip-F31-chain3
EVTLKESGPVLVKPTETLTLTCTVSGFSLTRYGINWIRQPPGKGLEWLGVIWTGGDTNYNSALKSRLTISKDKSKSQVVLTMTNMDPVDTATYYCAREGVVNYYGSRYSFFDVWGQGTTVTVSSASTKGPSVFPLAPSSKSTSGGTAALGCLVKDYFPEPVTVSWNSGALTSGVHTFPAVLQSSGLYSLSSVVTVPSSSLGTQTYICNVNHKPSNTKVDKKVEPKSCDKTHTCPPCPAPELLGGPSVFLFPPKPKDTLMISRTPEVTCVVVDVSHEDPEVKFNWYVDGVEVHNAKTKPREEQYNSTYRVVSVLTVLHQDWLNGKEYKCKVSNKALPAPIEKTISKAKGQPREPQVYTLPPCRDELTKNQVSLWCLVKGFYPSDIAVEWESNGQPENNYKTTPPVLDSDGSFFLYSKLTVDKSRWQQGNVFSCSVMHEALHNHYTQKSLSLSPGK

SEQ ID NO: 10 - protein, 213 aa, synthetic construct; identical to SEQ ID NO: 4
  CHAIN 1..213: note = CP11-Ip-F31-chain4

SEQ ID NO: 11 - protein, 355 aa, Homo sapiens
  CHAIN 1..355: note = CCR8
MDYTLDLSVTTVTDYYYPDIFSSPCDAELIQTNGKLLLAVFYCLLFVFSLLGNSLVILVLVVCKKLRSITDVYLLNLALSDLLFVFSFPFQTYYLLDQWVFGTVMCKVVSGFYYIGFYSSMFFITLMSVDRYLAVVHAVYALKVRTIRMGTTLCLAVWLTAIMATIPLLVFYQVASEDGVLQCYSFYNQQTLKWKIFTNFKMNILGLLIPFTIFMFCYIKILHQLKRCQNHNKTKAIRLVLIVVIASLLFWVPFNVVLFLTSLHSMHILDGCSISQQLTYATHVTEIISFTHCCVNPVIYAFVGEKFKKHLSEIFQKSCSQIFNYLGRQMPRESCEKSSSCQQHSSRSSSVDYIL

SEQ ID NO: 12 - protein, 394 aa, synthetic construct
  CHAIN 1..394: note = CTLA4-Fc
MACLGFQRHKAQLNLATRTWPCTLLFFLLFIPVFCKAMHVAQPAVVLASSRGIASFVCEYASPGKATEVRVTVLRQADSQVTEVCAATYMMGNELTFLDDSICTGTSSGNQVNLTIQGLRAMDTGLYICKVELMYPPPYYLGIGNGTQIYVIDPEPCPDSDFGGGGSDKTHTCPPCPAPELLGGPSVFLFPPKPKDTLMISRTPEVTCVVVDVSHEDPEVKFNWYVDGVEVHNAKTKPREEQYNSTYRVVSVLTVLHQDWLNGKEYKCKVSNKALPAPIEKTISKAKGQPREPQVYTLPPSRDELTKNQVSLTCLVKGFYPSDIAVEWESNGQPENNYKTTPPVLDSDGSFFLYSKLTVDKSRWQQGNVFSCSVMHEALHNHYTQKSLSLSPGK

SEQ ID NO: 13 - protein, 124 aa, synthetic construct
  REGION 1..124: note = CP11-VH
EVTLKESGPVLVKPTETLTLTCTVSGFSLTRYGINWIRQPPGKGLEWLGVIWTGGDTNYNSALKSRLTISKDKSKSQVVLTMTNMDPVDTATYYCAREGVVNYYGSRYSFFDVWGQGTTVTVSS

SEQ ID NO: 14 - protein, 106 aa, synthetic construct
  REGION 1..106: note = CP11-VL
DIQMTQSPSSLSASVGDRVTITCRASSSVSYMHWYQQKPGKSPKPWIYATSNLASGVPSRFSGSGSGTDYTLTISSLQPEDFATYYCQQWSSNPYTFGGGTKVEIK

SEQ ID NO: 15 - protein, 450 aa, synthetic construct
  CHAIN 1..450: note = Trastuzumab-heavy chain
EVQLVESGGGLVQPGGSLRLSCAASGFNIKDTYIHWVRQAPGKGLEWVARIYPTNGYTRYADSVKGRFTISADTSKNTAYLQMNSLRAEDTAVYYCSRWGGDGFYAMDYWGQGTLVTVSSASTKGPSVFPLAPSSKSTSGGTAALGCLVKDYFPEPVTVSWNSGALTSGVHTFPAVLQSSGLYSLSSVVTVPSSSLGTQTYICNVNHKPSNTKVDKKVEPKSCDKTHTCPPCPAPELLGGPSVFLFPPKPKDTLMISRTPEVTCVVVDVSHEDPEVKFNWYVDGVEVHNAKTKPREEQYNSTYRVVSVLTVLHQDWLNGKEYKCKVSNKALPAPIEKTISKAKGQPREPQVYTLPPSREEMTKNQVSLTCLVKGFYPSDIAVEWESNGQPENNYKTTPPVLDSDGSFFLYSKLTVDKSRWQQGNVFSCSVMHEALHNHYTQKSLSLSPGK

SEQ ID NO: 16 - protein, 214 aa, synthetic construct
  CHAIN 1..214: note = Trastuzumab-light chain
DIQMTQSPSSLSASVGDRVTITCRASQDVNTAVAWYQQKPGKAPKLLIYSASFLYSGVPSRFSGSRSGTDFTLTISSLQPEDFATYYCQQHYTTPPTFGQGTKVEIKRTVAAPSVFIFPPSDEQLKSGTASVVCLLNNFYPREAKVQWKVDNALQSGNSQESVTEQDSKDSTYSLSSTLTLSKADYEKHKVYACEVTHQGLSSPVTKSFNRGEC

SEQ ID NO: 17 - protein, 449 aa, synthetic construct
  CHAIN 1..449: note = Pertuzumab-heavy chain
EVQLVESGGGLVQPGGSLRLSCAASGFTFTDYTMDWVRQAPGKGLEWVADVNPNSGGSIYNQRFKGRFTLSVDRSKNTLYLQMNSLRAEDTAVYYCARNLGPSFYFDYWGQGTLVTVSSASTKGPSVFPLAPSSKSTSGGTAALGCLVKDYFPEPVTVSWNSGALTSGVHTFPAVLQSSGLYSLSSVVTVPSSSLGTQTYICNVNHKPSNTKVDKKVEPKSCDKTHTCPPCPAPELLGGPSVFLFPPKPKDTLMISRTPEVTCVVVDVSHEDPEVKFNWYVDGVEVHNAKTKPREEQYNSTYRVVSVLTVLHQDWLNGKEYKCKVSNKALPAPIEKTISKAKGQPREPQVYTLPPSREEMTKNQVSLTCLVKGFYPSDIAVEWESNGQPENNYKTTPPVLDSDGSFFLYSKLTVDKSRWQQGNVFSCSVMHEALHNHYTQKSLSLSPGK

SEQ ID NO: 18 - protein, 214 aa, synthetic construct
  CHAIN 1..214: note = Pertuzumab-light chain
DIQMTQSPSSLSASVGDRVTITCKASQDVSIGVAWYQQKPGKAPKLLIYSASYRYTGVPSRFSGSGSGTDFTLTISSLQPEDFATYYCQQYYIYPYTFGQGTKVEIKRTVAAPSVFIFPPSDEQLKSGTASVVCLLNNFYPREAKVQWKVDNALQSGNSQESVTEQDSKDSTYSLSSTLTLSKADYEKHKVYACEVTHQGLSSPVTKSFNRGEC

SEQ ID NO: 19 - protein, 125 aa, synthetic construct
  DOMAIN 1..125: note = Anti-CD3-VH
EVKLLESGGGLVQPKGSLKLSCAASGFTFNTYAMNWVRQAPGKGLEWVARIRSKYNNYATYYADSVKDRFTISRDDSQSILYLQMNNLKTEDTAMYYCVRHGNFGNSYVSWFAYWGQGTLVTVSA

SEQ ID NO: 20 - protein, 109 aa, synthetic construct
  DOMAIN 1..109: note = Anti-CD3-VL
QAVVTQESALTTSPGETVTLTCRSSTGAVTTSNYANWVQEKPDHLFTGLIGGTNKRAPGVPARFSGSLIGDKAALTITGAQTEDEAIYFCALWYSNLWVFGGGTKLTVL

SEQ ID NO: 21 - protein, 5 aa, synthetic construct
  REGION 1..5: note = CD3-HCDR1
TYAMN

SEQ ID NO: 22 - protein, 19 aa, synthetic construct
  REGION 1..19: note = CD3-HCDR2
RIRSKYNNYATYYADSVKD

SEQ ID NO: 23 - protein, 14 aa, synthetic construct
  REGION 1..14: note = CD3-HCDR3
HENFGQSYVSWFAY

SEQ ID NO: 24 - protein, 14 aa, synthetic construct
  REGION 1..14: note = CD3-LCDR1
ASSTGAVTTSNYPN

SEQ ID NO: 25 - protein, 7 aa, synthetic construct
  REGION 1..7: note = CD3-LCDR2
GTNKRAP

SEQ ID NO: 26 - protein, 9 aa, synthetic construct
  REGION 1..9: note = CD3-LCDR3
ALWYSELWV

SEQ ID NO: 27 - protein, 125 aa, synthetic construct
  DOMAIN 1..125: note = Anti-CD3-Hu-VH
EVQLLESGGGLVQPGGSLRLSCAASGFTFSTYAMNWVRQAPGKGLEWVSRIRSKYNNYATYYADSVKDRFTISRDDSKNTLYLQMNSLRAEDTAVYYCARHENFGQSYVSWFAYWGQGTTVTVSS

SEQ ID NO: 28 - protein, 109 aa, synthetic construct
  DOMAIN 1..109: note = Anti-CD3-Hu-VL
QTVVTQEPSLTVSPGGTVTLTCASSTGAVTTSNYPNWVQQKPGQAPRGLIGGTNKRAPGVPARFSGSLLGGKAALTLSGVQPEDEAEYYCALWYSELWVFGGGTKLTVL

SEQ ID NO: 29 - protein, 330 aa, synthetic construct
  CHAIN 1..330: note = IgG1-LALAGA
ASTKGPSVFPLAPSSKSTSGGTAALGCLVKDYFPEPVTVSWNSGALTSGVHTFPAVLQSSGLYSLSSVVTVPSSSLGTQTYICNVNHKPSNTKVDKKVEPKSCDKTHTCPPCPAPEAAGAPSVFLFPPKPKDTLMISRTPEVTCVVVDVSHEDPEVKFNWYVDGVEVHNAKTKPREEQYNSTYRVVSVLTVLHQDWLNGKEYKCKVSNKALPAPIEKTISKAKGQPREPQVYTLPPSREEMTKNQVSLTCLVKGFYPSDIAVEWESNGQPENNYKTTPPVLDSDGSFFLYSKLTVDKSRWQQGNVFSCSVMHEALHNHYTQKSLSLSPGK

SEQ ID NO: 30 - protein, 106 aa, synthetic construct
  DOMAIN 1..106: note = Lambda-CL
GQPKAAPSVTLFPPSSEELQANKATLVCLISDFYPGAVTVAWKADSSPVKAGVETTTPSKQSNNKYAASSYLSLTPEQWKSHRSYSCQVTHEGSTVEKTVAPTECS

SEQ ID NO: 31 - protein, 455 aa, synthetic construct
  CHAIN 1..455: note = Anti-CD3-Hu-HC
EVQLLESGGGLVQPGGSLRLSCAASGFTFSTYAMNWVRQAPGKGLEWVSRIRSKYNNYATYYADSVKDRFTISRDDSKNTLYLQMNSLRAEDTAVYYCARHENFGQSYVSWFAYWGQGTTVTVSSASTKGPSVFPLAPSSKSTSGGTAALGCLVKDYFPEPVTVSWNSGALTSGVHTFPAVLQSSGLYSLSSVVTVPSSSLGTQTYICNVNHKPSNTKVDKKVEPKSCDKTHTCPPCPAPEAAGAPSVFLFPPKPKDTLMISRTPEVTCVVVDVSHEDPEVKFNWYVDGVEVHNAKTKPREEQYNSTYRVVSVLTVLHQDWLNGKEYKCKVSNKALPAPIEKTISKAKGQPREPQVYTLPPSREEMTKNQVSLTCLVKGFYPSDIAVEWESNGQPENNYKTTPPVLDSDGSFFLYSKLTVDKSRWQQGNVFSCSVMHEALHNHYTQKSLSLSPGK

SEQ ID NO: 32 - protein, 215 aa, synthetic construct
  CHAIN 1..215: note = Anti-CD3-Hu-LC
QTVVTQEPSLTVSPGGTVTLTCASSTGAVTTSNYPNWVQQKPGQAPRGLIGGTNKRAPGVPARFSGSLLGGKAALTLSGVQPEDEAEYYCALWYSELWVFGGGTKLTVLGQPKAAPSVTLFPPSSEELQANKATLVCLISDFYPGAVTVAWKADSSPVKAGVETTTPSKQSNNKYAASSYLSLTPEQWKSHRSYSCQVTHEGSTVEKTVAPTECS

SEQ ID NO: 33 - protein, 447 aa, synthetic construct
  CHAIN 1..447: note = Hu67-14-HC
EVQLVQSGAEVKKPGESLKISCKGSGYSFTDYHMNWVKQMPGKGLEWMGDINPDIGGTSYNQNFKGKVTISVDKSISTAYLQWSSLKASDTAMYYCARWDFDSFANWGQGTLVTVSSASTKGPSVFPLAPSSKSTSGGTAALGCLVKDYFPEPVTVSWNSGALTSGVHTFPAVLQSSGLYSLSSVVTVPSSSLGTQTYICNVNHKPSNTKVDKKVEPKSCDKTHTCPPCPAPELLGGPSVFLFPPKPKDTLMISRTPEVTCVVVDVSHEDPEVKFNWYVDGVEVHNAKTKPREEQYNSTYRVVSVLTVLHQDWLNGKEYKCKVSNKALPAPIEKTISKAKGQPREPQVYTLPPSRDELTKNQVSLTCLVKGFYPSDIAVEWESNGQPENNYKTTPPVLDSDGSFFLYSKLTVDKSRWQQGNVFSCSVMHEALHNHYTQKSLSLSPGK

SEQ ID NO: 34 - protein, 218 aa, synthetic construct
  CHAIN 1..218: note = Hu67-14-LC
DIQMTQSPSSLSASVGDRVTITCRASESVSIIGTNLIHWYQQKPGKAPKLLIYHASNLETGVPSRFSGSGSGTDFTLTISSLQPEDFATYYCLQSRKIPYTFGGGTKVEIKRTVAAPSVFIFPPSDEQLKSGTASVVCLLNNFYPREAKVQWKVDNALQSGNSQESVTEQDSKDSTYSLSSTLTLSKADYEKHKVYACEVTHQGLSSPVTKSFNRGEC

SEQ ID NO: 35 - protein, 453 aa, synthetic construct
  CHAIN 1..453: note = M6H2L2-HC
EVQLVQSGAEVKKPGASVKVSCKASGYRFIPYWIEWVRQAPGQGLEWMGEILPGTGRTNYNEKFKGRVTFTADTSTNTVYMELSSLRSEDTAVYYCARYGDDTSGGYYAVDYWGQGTTVTVSSASTKGPSVFPLAPSSKSTSGGTAALGCLVKDYFPEPVTVSWNSGALTSGVHTFPAVLQSSGLYSLSSVVTVPSSSLGTQTYICNVNHKPSNTKVDKKVEPKSCDKTHTCPPCPAPELLGGPSVFLFPPKPKDTLMISRTPEVTCVVVDVSHEDPEVKFNWYVDGVEVHNAKTKPREEQYNSTYRVVSVLTVLHQDWLNGKEYKCKVSNKALPAPIEKTISKAKGQPREPQVYTLPPSRDELTKNQVSLTCLVKGFYPSDIAVEWESNGQPENNYKTTPPVLDSDGSFFLYSKLTVDKSRWQQGNVFSCSVMHEALHNHYTQKSLSLSPGK

SEQ ID NO: 36 - protein, 218 aa, synthetic construct
  CHAIN 1..218: note = M6H2L2-LC
EIVLTQSPATLSLSPGERATLSCRASESVNILGTNLIHWYQQKPGQAPKLLIYHASNLETGIPARFSGSGSRTDFTLTISSLEPEDFAVYYCLQSRKIPWTFGGGTKVEIKRTVAAPSVFIFPPSDEQLKSGTASVVCLLNNFYPREAKVQWKVDNALQSGNSQESVTEQDSKDSTYSLSSTLTLSKADYEKHKVYACEVTHQGLSSPVTKSFNRGEC

SEQ ID NO: 37 - protein, 690 aa, synthetic construct
  CHAIN 1..690: note = Anti-CEA*MUC1-HC
EVQLVQSGAEVKKPGASVKVSCKASGYRFIPYWIEWVRQAPGQGLEWMGEILPGTGRTNYNEKFKGRVTFTADTSTNTVYMELSSLRSEDTAVYYCARYGDDTSGGYYAVDYWGEGTTVTVSSASTKGPSVFPLAPSSKSTSGGTAALGCLVKDYFPEPVTVSWNSGALTSGVHTFPAVLQSSGLYSLSSVVTVPSSSLGTQTYICNVNHKPSNTKVDKKVEPKSCDKGGGGSGGGGSGGGGSEVQLVQSGAEVKKPGESLKISCKGSGYSFTDYHMNWVKQMPGKGLEWMGDINPDIGGTSYNQNFKGKVTISVDKSISTAYLQWSSLKASDTAMYYCARWDFDSFANWGEGTLVTVSSASTKGPSVFPLAPSSKSTSGGTAALGCLVKDYFPEPVTVSWNSGALTSGVHTFPAVLQSSGLYSLSSVVTVPSSSLGTQTYICNVNHKPSNTKVDKKVEPKSCDKTHTCPPCPAPEAAGAPSVFLFPPKPKDTLMISRTPEVTCVVVDVSHEDPEVKFNWYVDGVEVHNAKTKPREEQYNSTYRVVSVLTVLHQDWLNGKEYKCKVSNKALPAPIEKTISKAKGQPREPQVYTLPPSREEMTKNQVSLTCLVKGFYPSDIAVEWESNGQPENNYKTTPPVLDSDGSFFLYSKLTVDKSRWQQGNVFSCSVMHEALHNHYTQKSLSLSPGK

SEQ ID NO: 38 - protein, 218 aa, synthetic construct
  CHAIN 1..218: note = Anti-CEA*MUC1-LC
DIQMTQSPSSLSASVGDRVTITCRASESVSIIGTNLIHWYQQKPGEAPKLLIYHASNLETGVPSRFSGSGSGTDFTLTISSLQPEDFATYYCLQSRKIPYTFGGGTKVEIKRTVAAPSVFIFPPSDEQLKSGTASVVCLLNNFYPREAKVQWKVDNALQSGNSQESVTEQDSKDSTYSLSSTLTLSKADYEKHKVYACEVTHQGLSSPVTKSFNRGEC

SEQ ID NO: 39 - protein, 330 aa, Homo sapiens
  CHAIN 1..330: note = hIgG1-1
ASTKGPSVFPLAPSSKSTSGGTAALGCLVKDYFPEPVTVSWNSGALTSGVHTFPAVLQSSGLYSLSSVVTVPSSSLGTQTYICNVNHKPSNTKVDKRVEPKSCDKTHTCPPCPAPELLGGPSVFLFPPKPKDTLMISRTPEVTCVVVDVSHEDPEVKFNWYVDGVEVHNAKTKPREEQYNSTYRVVSVLTVLHQDWLNGKEYKCKVSNKALPAPIEKTISKAKGQPREPQVYTLPPSRDELTKNQVSLTCLVKGFYPSDIAVEWESNGQPENNYKTTPPVLDSDGSFFLYSKLTVDKSRWQQGNVFSCSVMHEALHNHYTQKSLSLSPGK

SEQ ID NO: 40 - protein, 330 aa, Homo sapiens [sequence omitted]

SEQ ID NO: 41 - protein, 330 aa, Homo sapiens
  CHAIN 1..330: note = hIgG1-3
ASTKGPSVFPLAPSSKSTSGGTAALGCLVKDYFPEPVTVSWNSGALTSGVHTFPAVLQSSGLYSLSSVVTVPSSSLGTQTYICNVNHKPSNTKVDKKVEPKSCDKTHTCPPCPAPELLGGPSVFLFPPKPKDTLMISRTPEVTCVVVDVSHEDPEVKFNWYVDGVEVHNAKTKPREEQYNSTYRVVSVLTVLHQDWLNGKEYKCKVSNKALPAPIEKTISKAKGQPREPQVYTLPPSREEMTKNQVSLTCLVKGFYPSDIAVEWESNGQPENNYKTTPPVLDSDGSFFLYSKLTVDKSRWQQGNVFSCSVMHEALHNHYTQKSLSLSPGK